European Patent Application EP 4 317 181 A1, published February 7, 2024. Title: Recombinant Type-I Humanized Collagen Polypeptide, and Preparation Method therefor and Use thereof. Applicant: SHANXI JINBO BIO-PHARMACEUTICAL CO., LTD. The sequence listing filed with the application follows.

SEQUENCE LISTING (18 sequences)

SEQ ID NO: 1 - protein, 60 aa, Artificial Sequence
  Unit of Repeat sequence
GEKGSPGADGPAGAPGTPGPQGIAGQRGVVGLPGQRGERGFPGLPGPSGEPGKQGPSGAS

SEQ ID NO: 2 - protein, 10 aa, Artificial Sequence
  Amino acid sequence of hinge region
GPPGPCCGGG

SEQ ID NO: 3 - protein, 240 aa, Artificial Sequence
  Amino acid sequence of TC1R4
GEKGSPGADGPAGAPGTPGPQGIAGQRGVVGLPGQRGERGFPGLPGPSGEPGKQGPSGASGEKGSPGADGPAGAPGTPGPQGIAGQRGVVGLPGQRGERGFPGLPGPSGEPGKQGPSGASGEKGSPGADGPAGAPGTPGPQGIAGQRGVVGLPGQRGERGFPGLPGPSGEPGKQGPSGASGEKGSPGADGPAGAPGTPGPQGIAGQRGVVGLPGQRGERGFPGLPGPSGEPGKQGPSGAS

SEQ ID NO: 4 - protein, 6 aa, Artificial Sequence
  Sequences cleaved off by TEV protease
ENLYFQ

SEQ ID NO: 5 - protein, 246 aa, Artificial Sequence
  Amino acid sequence of TC1R4 with sequence that can be cleaved off by TEV protease
ENLYFQGEKGSPGADGPAGAPGTPGPQGIAGQRGVVGLPGQRGERGFPGLPGPSGEPGKQGPSGASGEKGSPGADGPAGAPGTPGPQGIAGQRGVVGLPGQRGERGFPGLPGPSGEPGKQGPSGASGEKGSPGADGPAGAPGTPGPQGIAGQRGVVGLPGQRGERGFPGLPGPSGEPGKQGPSGASGEKGSPGADGPAGAPGTPGPQGIAGQRGVVGLPGQRGERGFPGLPGPSGEPGKQGPSGAS

SEQ ID NO: 6 - DNA, 753 bp, Artificial Sequence
  The DNA sequence of TC1R4 comprising the restriction site, stop codon and sequence that can be cleaved off by TEV protease
ggtaccgaaaacctgtatttccagggtgaaaaaggtagtccgggtgcagatggtccggccggtgcacctggtacaccgggtcctcagggcattgcaggccagcgtggtgttgtgggcctgccgggtcagcgcggtgaacgtggttttccgggtctgccgggtccgagcggcgaacctggtaaacagggcccgagtggtgcaagcggtgaaaaaggcagtccgggcgcagatggtcctgcaggtgcccctggtacacctggtccgcagggtattgcaggtcagcgcggcgtggtgggcctgcctggtcaacgtggcgaacgtggtttcccgggcctgccgggaccgtcaggtgaacctggcaaacagggccctagcggtgcaagtggcgaaaaaggtagcccgggcgcagacggcccggcaggtgcacctggcacacctggtcctcagggtattgcgggccagcgcggcgttgttggtctgcctggccagcgtggcgaacgcggttttccgggcctgcctggcccgtcaggcgaacctggaaaacagggcccaagtggtgcaagtggtgaaaaaggaagtccgggcgccgatggcccggccggtgcgcctggtacgcctggtcctcaaggcattgccggtcagcgcggagttgttggcctgccgggccagcgtggagaacgcggtttcccgggtctgcctggtccgagtggtgaaccgggtaaacagggtccgagcggtgcatcataactcgag

SEQ ID NO: 7 - protein, 18 aa, Artificial Sequence
  Partial sequence of mass spectrometry detection result of TC1R4
ADGAILVDFWAEWCGPCK

SEQ ID NO: 8 - protein, 27 aa, Artificial Sequence
  Partial sequence of mass spectrometry detection result of TC1R4
GERGFPGLPGPSGEPGKQGPSGASGEK

SEQ ID NO: 9 - protein, 24 aa, Artificial Sequence
  Partial sequence of mass spectrometry detection result of TC1R4
GFPGLPGPSGEPGKQGPSGASGEK

SEQ ID NO: 10 - protein, 51 aa, Artificial Sequence
  Partial sequence of mass spectrometry detection result of TC1R4
GERGFPGLPGPSGEPGKQGPSGASGEKGSPGADGPAGAPGTPGPQGIAGQR

SEQ ID NO: 11 - protein, 34 aa, Artificial Sequence
  Partial sequence of mass spectrometry detection result of TC1R4
QGPSGASGEKGSPGADGPAGAPGTPGPQGIAGQR

SEQ ID NO: 12 - protein, 24 aa, Artificial Sequence
  Partial sequence of mass spectrometry detection result of TC1R4
GSPGADGPAGAPGTPGPQGIAGQR

SEQ ID NO: 13 - protein, 9 aa, Artificial Sequence
  Partial sequence of mass spectrometry detection result of TC1R4
GVVGLPGQR

SEQ ID NO: 14 - protein, 12 aa, Artificial Sequence
  Partial sequence of mass spectrometry detection result of TC1R4
GVVGLPGQRGER

SEQ ID NO: 15 - protein, 17 aa, Artificial Sequence
  Partial sequence of mass spectrometry detection result of TC1R4
GERGFPGLPGPSGEPGK

SEQ ID NO: 16 - protein, 24 aa, Artificial Sequence
  Partial sequence of mass spectrometry detection result of TC1R4
GERGFPGLPGPSGEPGKQGPSGAS

SEQ ID NO: 17 - protein, 14 aa, Artificial Sequence
  Partial sequence of mass spectrometry detection result of TC1R4
GFPGLPGPSGEPGK

SEQ ID NO: 18 - protein, 21 aa, Artificial Sequence
  Partial sequence of mass spectrometry detection result of TC1R4
GFPGLPGPSGEPGKQGPSGAS